European Patent Application EP 4 163 300 A1, published April 12, 2023. Title: Anti-GFRAL antibody and use thereof. Applicant: Daegu Gyeongbuk Institute of Science and Technology. The sequence listing filed with the application follows.

SEQUENCE LISTING (24 sequences)

SEQ ID NO: 1 - protein, 8 aa, Artificial Sequence
  A8 VH CDR1
GFTFDDYA

SEQ ID NO: 2 - protein, 8 aa, Artificial Sequence
  A8 VH CDR2
ISWNSGNI

SEQ ID NO: 3 - protein, 15 aa, Artificial Sequence
  A8 VH CDR3
CAKDISYGSGSSFDY

SEQ ID NO: 4 - protein, 9 aa, Artificial Sequence
  A8 VL CDR1
SSDVGGYNY

SEQ ID NO: 5 - protein, 3 aa, Artificial Sequence
  A8 VL CDR2
GVT

SEQ ID NO: 6 - protein, 10 aa, Artificial Sequence
  A8 VL CDR3
LSYAGSYNWV

SEQ ID NO: 7 - protein, 8 aa, Artificial Sequence
  A11 VH CDR1
GFTFSSYG

SEQ ID NO: 8 - protein, 8 aa, Artificial Sequence
  A11 VH CDR2
ISYDGSNK

SEQ ID NO: 9 - protein, 21 aa, Artificial Sequence
  A11 VH CDR3
CAKVTSGGDFWSGNYYYYMDV

SEQ ID NO: 10 - protein, 6 aa, Artificial Sequence
  A11 VL CDR1
SLRDYY

SEQ ID NO: 11 - protein, 3 aa, Artificial Sequence
  A11 VL CDR2
GKN

SEQ ID NO: 12 - protein, 10 aa, Artificial Sequence
  A11 VL CDR3
NSRGSSNQWV

SEQ ID NO: 13 - protein, 8 aa, Artificial Sequence
  B9 VH CDR1
GGTFSSYA

SEQ ID NO: 14 - protein, 8 aa, Artificial Sequence
  B9 VH CDR2
IIPIFGTA

SEQ ID NO: 15 - protein, 18 aa, Artificial Sequence
  B9 VH CDR3
CARPMDRYSLTTPLAFDI

SEQ ID NO: 16 - protein, 9 aa, Artificial Sequence
  B9 VL CDR1
SSDVGGYDY

SEQ ID NO: 17 - protein, 3 aa, Artificial Sequence
  B9 VL CDR2
EVS

SEQ ID NO: 18 - protein, 10 aa, Artificial Sequence
  B9 VL CDR3
SSYAGSNDLV

SEQ ID NO: 19 - protein, 8 aa, Artificial Sequence
  D12 VH CDR1
GYTFTGYY

SEQ ID NO: 20 - protein, 8 aa, Artificial Sequence
  D12 VH CDR2
INPNSGGT

SEQ ID NO: 21 - protein, 14 aa, Artificial Sequence
  D12 VH CDR3
CAKDQWLGHYGMDV

SEQ ID NO: 22 - protein, 6 aa, Artificial Sequence
  D12 VL CDR1
QGISSS

SEQ ID NO: 23 - protein, 3 aa, Artificial Sequence
  D12 VL CDR2
AAS

SEQ ID NO: 24 - protein, 9 aa, Artificial Sequence
  D12 VL CDR3
QQTYHTPQT